European Patent Application EP 4 696 715 A1, published February 18, 2026. Title: 抗CTLA4-抗PD-1双特异性抗体的医药用途. Applicant: 康方药业有限公司. The sequence listing filed with the application follows.

SEQUENCE LISTING (47 sequences)

SEQ ID NO: 1 - DNA, 372 bp, synthetic construct
  source 1..372: mol_type = other DNA
caggtcaagctgcaggagtctggacctgagctggtgaagcctggagcttcaatgaagatatcctgcaaggcttctggttactcattcactggctacaccatgaactgggtgaagcagagccatggaaagaaccttgaatggattggacttattaatccttacaataatattactaactacaaccagaagttcatgggcaaggccacatttactgtagacaagtcatccagcacagcctacatggaactcctcagactgacatctgaagactctggagtctatttctgtgcaagactcgactataggtcttattggggccaagggactctggtcactgtctctgcagccaaaacgacacccccatctgtctat

SEQ ID NO: 2 - protein, 124 aa, synthetic construct
QVKLQESGPELVKPGASMKISCKASGYSFTGYTMNWVKQSHGKNLEWIGLINPYNNITNYNQKFMGKATFTVDKSSSTAYMELLRLTSEDSGVYFCARLDYRSYWGQGTLVTVSAAKTTPPSVY

SEQ ID NO: 3 - DNA, 378 bp, synthetic construct
  source 1..378: mol_type = other DNA
caggctgttgtgactcaggaatctgcactcaccacatcacctggtgaaacagtcacactcacttgtcgctcaagtactggggctgttacaactagtaactttgccaactgggtccaagaaaaaccagatcatttattcactagtctaataggtggtaccaacaaccgagctccaggtgttcctgccagattctcaggctccctgattggagacaaggctgccctcaccatcacaggggcacagactgaggatgaggcaatatatttctgtgctctatggtacagcaaccattgggtgttcggtggaggaaccaaactgactgtcctaggccagcccaagtcttcgccatcagtcaccctgtttcaagggcaattctgc

SEQ ID NO: 4 - protein, 126 aa, synthetic construct
QAVVTQESALTTSPGETVTLTCRSSTGAVTTSNFANWVQEKPDHLFTSLIGGTNNRAPGVPARFSGSLIGDKAALTITGAQTEDEAIYFCALWYSNHWVFGGGTKLTVLGQPKSSPSVTLFQGQFC

SEQ ID NO: 5 - DNA, 345 bp, synthetic construct
  source 1..345: mol_type = other DNA
caggtgcagctggtggagtctggggccgagctggtgaagcccggcgcctccatgaagatctcttgcaaggccagcggatacagtttcactggctataccatgaactgggtcaaacaggctccaggacagggactggagtggatcgggctgattaatccttacaacaacatcaccaactacaaccagaagttcatgggaaaagcaacctttacagtggacaagagcatttccacagcctacatggaactgagccggctgacttcagacgatagcggggtctatttttgtgcaaggctggattatcgctcttactgggggcagggaactctggtcactgtctccgct

SEQ ID NO: 6 - protein, 115 aa, synthetic construct
QVQLVESGAELVKPGASMKISCKASGYSFTGYTMNWVKQAPGQGLEWIGLINPYNNITNYNQKFMGKATFTVDKSISTAYMELSRLTSDDSGVYFCARLDYRSYWGQGTLVTVSA

SEQ ID NO: 7 - DNA, 327 bp, synthetic construct
  source 1..327: mol_type = other DNA
caggctgtcgtcactcaggaaccttcactgactgtgagcccaggaggaactgtcaccctgacatgcggaagctccaccggagcagtgaccacatccaacttcgccaattgggtccaggaaaagccaggccaggcatttcgatccctgatcggaggcacaaacaatcgggcttcttgggtgcccgcaagattctcaggaagcctgctggggggaaaagccgctctgaccattagtggcgctcagcctgaggacgaagccgagtacttctgcgctctgtggtatagcaaccactgggtgtttggcgggggaacaaagctgactgtgctg

SEQ ID NO: 8 - protein, 109 aa, synthetic construct
QAVVTQEPSLTVSPGGTVTLTCGSSTGAVTTSNFANWVQEKPGQAFRSLIGGTNNRASWVPARFSGSLLGGKAALTISGAQPEDEAEYFCALWYSNHWVFGGGTKLTVL

SEQ ID NO: 9 - DNA, 345 bp, synthetic construct
  source 1..345: mol_type = other DNA
caggtgcagctggtcgagtctggggccgaagtgaagaaacccggcgcctcagtgaaggtcagctgcaaggccagcgggtacagtttcactggatataccatgaactgggtccgacaggcccctggccaggggctggagtggatcggcctgattaacccttacaacaacatcactaactacgcacagaagttccaggggagagtgacctttacagtggacaccagcatttccacagcctacatggaactgtcccggctgagatctgacgatacaggcgtgtacttctgcgctaggctggattaccgcagctattggggacagggcacactggtgactgtcagcgca

SEQ ID NO: 10 - protein, 115 aa, synthetic construct
QVQLVESGAEVKKPGASVKVSCKASGYSFTGYTMNWVRQAPGQGLEWIGLINPYNNITNYAQKFQGRVTFTVDTSISTAYMELSRLRSDDTGVYFCARLDYRSYWGQGTLVTVSA

SEQ ID NO: 11 - DNA, 327 bp, synthetic construct
  source 1..327: mol_type = other DNA
caggctgtcgtcactcaggaaccttcactgaccgtgtctcctggcgggactgtcaccctgacatgcggcagctccacaggggccgtgaccacaagtaacttcccaaattgggtccagcagaagccaggacaggctccccggagtctgatcggaggcaccaacaacaaggccagctggacacccgcacggttcagcggcagcctgctgggcggcaaggccgctctgacaattagcggagcccagcctgaggacgaagccgagtactattgcgctctgtggtactccaaccactgggtgttcggcggcggcaccaagctgactgtgctg

SEQ ID NO: 12 - protein, 109 aa, synthetic construct
QAVVTQEPSLTVSPGGTVTLTCGSSTGAVTTSNFPNWVQQKPGQAPRSLIGGTNNKASWTPARFSGSLLGGKAALTISGAQPEDEAEYYCALWYSNHWVFGGGTKLTVL

SEQ ID NO: 13 - DNA, 354 bp, synthetic construct
  source 1..354: mol_type = other DNA
gaggtcaaactggtggagagcggcggcgggctggtgaagcccggcgggtcactgaaactgagctgcgccgcttccggcttcgcctttagctcctacgacatgtcatgggtgaggcagacccctgagaagcgcctggaatgggtcgctactatcagcggaggcgggcgatacacctactatcctgactctgtcaaagggagattcacaattagtcgggataacgccagaaatactctgtatctgcagatgtctagtctgcggtccgaggatacagctctgtactattgtgcaaaccggtacggcgaagcatggtttgcctattggggacagggcaccctggtgacagtctctgcc

SEQ ID NO: 14 - protein, 118 aa, synthetic construct
EVKLVESGGGLVKPGGSLKLSCAASGFAFSSYDMSWVRQTPEKRLEWVATISGGGRYTYYPDSVKGRFTISRDNARNTLYLQMSSLRSEDTALYYCANRYGEAWFAYWGQGTLVTVSA

SEQ ID NO: 15 - DNA, 321 bp, synthetic construct
  source 1..321: mol_type = other DNA
gacattaagatgacacagtccccttcctcaatgtacgctagcctgggcgagcgagtgaccttcacatgcaaagcatcccaggacatcaacacatacctgtcttggtttcagcagaagccaggcaaaagccccaagaccctgatctaccgggccaatagactggtggacggggtccccagcagattctccggatctggcagtgggcaggattactccctgaccatcagctccctggagtatgaagacatgggcatctactattgcctgcagtatgatgagttccctctgacctttggagcaggcacaaaactggaactgaag

SEQ ID NO: 16 - protein, 107 aa, synthetic construct
DIKMTQSPSSMYASLGERVTFTCKASQDINTYLSWFQQKPGKSPKTLIYRANRLVDGVPSRFSGSGSGQDYSLTISSLEYEDMGIYYCLQYDEFPLTFGAGTKLELK

SEQ ID NO: 17 - DNA, 354 bp, synthetic construct
  source 1..354: mol_type = other DNA
gaagtgcagctggtcgagtctgggggagggctggtgcagcccggcgggtcactgcgactgagctgcgcagcttccggattcgcctttagctcctacgacatgtcctgggtgcgacaggcaccaggaaagggactggattgggtcgctactatctcaggaggcgggagatacacctactatcctgacagcgtcaagggccggttcacaatctctagagataacagtaagaacaatctgtatctgcagatgaacagcctgagggctgaggacaccgcactgtactattgtgccaaccgctacggggaagcatggtttgcctattgggggcagggaaccctggtgacagtctctagt

SEQ ID NO: 18 - protein, 118 aa, synthetic construct
EVQLVESGGGLVQPGGSLRLSCAASGFAFSSYDMSWVRQAPGKGLDWVATISGGGRYTYYPDSVKGRFTISRDNSKNNLYLQMNSLRAEDTALYYCANRYGEAWFAYWGQGTLVTVSS

SEQ ID NO: 19 - DNA, 321 bp, synthetic construct
  source 1..321: mol_type = other DNA
gacattcagatgactcagagcccctcctccatgtccgcctctgtgggcgacagggtcaccttcacatgccgcgctagtcaggatatcaacacctacctgagctggtttcagcagaagccagggaaaagccccaagacactgatctaccgggctaatagactggtgtctggagtcccaagtcggttcagtggctcagggagcggacaggactacactctgaccatcagctccctgcagcctgaggacatggcaacctactattgcctgcagtatgatgagttcccactgacctttggcgccgggacaaaactggagctgaag

SEQ ID NO: 20 - protein, 107 aa, synthetic construct
DIQMTQSPSSMSASVGDRVTFTCRASQDINTYLSWFQQKPGKSPKTLIYRANRLVSGVPSRFSGSGSGQDYTLTISSLQPEDMATYYCLQYDEFPLTFGAGTKLELK

SEQ ID NO: 21 - DNA, 1344 bp, synthetic construct
  source 1..1344: mol_type = other DNA
gaagtgcagctggtcgagtctgggggagggctggtgcagcccggcgggtcactgcgactgagctgcgcagcttccggattcgcctttagctcctacgacatgtcctgggtgcgacaggcaccaggaaagggactggattgggtcgctactatctcaggaggcgggagatacacctactatcctgacagcgtcaagggccggttcacaatctctagagataacagtaagaacaatctgtatctgcagatgaacagcctgagggctgaggacaccgcactgtactattgtgccaaccgctacggggaagcatggtttgcctattgggggcagggaaccctggtgacagtctctagtgccagcaccaaaggacctagcgtgtttcctctcgccccctcctccaaaagcaccagcggaggaaccgctgctctcggatgtctggtgaaggactacttccctgaacccgtcaccgtgagctggaatagcggcgctctgacaagcggagtccatacattccctgctgtgctgcaaagcagcggactctattccctgtccagcgtcgtcacagtgcccagcagcagcctgggcacccagacctacatctgtaacgtcaaccacaagccctccaacaccaaggtggacaagaaagtggagcccaaatcctgcgacaagacacacacctgtcccccctgtcctgctcccgaactcctcggaggccctagcgtcttcctctttcctcccaaacccaaggacaccctcatgatcagcagaacccctgaagtcacctgtgtcgtcgtggatgtcagccatgaggaccccgaggtgaaattcaactggtatgtcgatggcgtcgaggtgcacaacgccaaaaccaagcccagggaggaacagtacaactccacctacagggtggtgtccgtgctgacagtcctccaccaggactggctgaacggcaaggagtacaagtgcaaggtgtccaacaaggctctccctgcccccattgagaagaccatcagcaaggccaaaggccaacccagggagccccaggtctatacactgcctccctccagggacgaactcaccaagaaccaggtgtccctgacctgcctggtcaagggcttttatcccagcgacatcgccgtcgagtgggagtccaacggacagcccgagaataactacaagaccacccctcctgtcctcgactccgacggctccttcttcctgtacagcaagctgaccgtggacaaaagcaggtggcagcagggaaacgtgttctcctgcagcgtgatgcacgaagccctccacaaccactacacccagaaaagcctgtccctgagccccggcaaa

SEQ ID NO: 22 - protein, 448 aa, synthetic construct
EVQLVESGGGLVQPGGSLRLSCAASGFAFSSYDMSWVRQAPGKGLDWVATISGGGRYTYYPDSVKGRFTISRDNSKNNLYLQMNSLRAEDTALYYCANRYGEAWFAYWGQGTLVTVSSASTKGPSVFPLAPSSKSTSGGTAALGCLVKDYFPEPVTVSWNSGALTSGVHTFPAVLQSSGLYSLSSVVTVPSSSLGTQTYICNVNHKPSNTKVDKKVEPKSCDKTHTCPPCPAPELLGGPSVFLFPPKPKDTLMISRTPEVTCVVVDVSHEDPEVKFNWYVDGVEVHNAKTKPREEQYNSTYRVVSVLTVLHQDWLNGKEYKCKVSNKALPAPIEKTISKAKGQPREPQVYTLPPSRDELTKNQVSLTCLVKGFYPSDIAVEWESNGQPENNYKTTPPVLDSDGSFFLYSKLTVDKSRWQQGNVFSCSVMHEALHNHYTQKSLSLSPGK

SEQ ID NO: 23 - DNA, 642 bp, synthetic construct
  source 1..642: mol_type = other DNA
gacattcagatgactcagagcccctcctccatgtccgcctctgtgggcgacagggtcaccttcacatgccgcgctagtcaggatatcaacacctacctgagctggtttcagcagaagccagggaaaagccccaagacactgatctaccgggctaatagactggtgtctggagtcccaagtcggttcagtggctcagggagcggacaggactacactctgaccatcagctccctgcagcctgaggacatggcaacctactattgcctgcagtatgatgagttcccactgacctttggcgccgggacaaaactggagctgaagcgaactgtggccgctccctccgtcttcatttttcccccttctgacgaacagctgaaatcaggcacagccagcgtggtctgtctgctgaacaatttctaccctagagaggcaaaagtgcagtggaaggtcgataacgccctgcagtccggcaacagccaggagagtgtgactgaacaggactcaaaagatagcacctattccctgtctagtacactgactctgtccaaggctgattacgagaagcacaaagtgtatgcatgcgaagtgacacatcagggactgtcaagccccgtgactaagtcttttaaccggggcgaatgt

SEQ ID NO: 24 - protein, 214 aa, synthetic construct
DIQMTQSPSSMSASVGDRVTFTCRASQDINTYLSWFQQKPGKSPKTLIYRANRLVSGVPSRFSGSGSGQDYTLTISSLQPEDMATYYCLQYDEFPLTFGAGTKLELKRTVAAPSVFIFPPSDEQLKSGTASVVCLLNNFYPREAKVQWKVDNALQSGNSQESVTEQDSKDSTYSLSSTLTLSKADYEKHKVYACEVTHQGLSSPVTKSFNRGEC

SEQ ID NO: 25 - protein, 15 aa, synthetic construct
GGGGSGGGGSGGGGS

SEQ ID NO: 26 - protein, 20 aa, synthetic construct
GGGGSGGGGSGGGGSGGGGS

SEQ ID NO: 27 - protein, 8 aa, synthetic construct
GFAFSSYD

SEQ ID NO: 28 - protein, 8 aa, synthetic construct
ISGGGRYT

SEQ ID NO: 29 - protein, 11 aa, synthetic construct
ANRYGEAWFAY

SEQ ID NO: 30 - protein, 6 aa, synthetic construct
QDINTY

SEQ ID NO: 31 - skipped

SEQ ID NO: 32 - protein, 9 aa, synthetic construct
LQYDEFPLT

SEQ ID NO: 33 - protein, 8 aa, synthetic construct
GYSFTGYT

SEQ ID NO: 34 - protein, 8 aa, synthetic construct
INPYNNIT

SEQ ID NO: 35 - protein, 8 aa, synthetic construct
ARLDYRSY

SEQ ID NO: 36 - protein, 9 aa, synthetic construct
TGAVTTSNF

SEQ ID NO: 37 - skipped

SEQ ID NO: 38 - protein, 9 aa, synthetic construct
ALWYSNHWV

SEQ ID NO: 39 - DNA, 1344 bp, synthetic construct
  source 1..1344: mol_type = other DNA
gaagtgcagctggtcgagtctgggggagggctggtgcagcccggcgggtcactgcgactgagctgcgcagcttccggattcgcctttagctcctacgacatgtcctgggtgcgacaggcaccaggaaagggactggattgggtcgctactatctcaggaggcgggagatacacctactatcctgacagcgtcaagggccggttcacaatctctagagataacagtaagaacaatctgtatctgcagatgaacagcctgagggctgaggacaccgcactgtactattgtgccaaccgctacggggaagcatggtttgcctattgggggcagggaaccctggtgacagtctctagtgccagcaccaaagggcccagcgtgtttcctctcgccccctcctccaaaagcaccagcggaggaaccgctgctctcggatgtctggtgaaggactacttccctgaacccgtcaccgtgagctggaatagcggcgctctgacaagcggagtccatacattccctgctgtgctgcaaagcagcggactctattccctgtccagcgtcgtcacagtgcccagcagcagcctgggcacccagacctacatctgtaacgtcaaccacaagccctccaacaccaaggtggacaagaaagtggagcccaaatcctgcgacaagacacacacctgtcccccctgtcctgctcccgaagctgctggagcccctagcgtcttcctctttcctcccaaacccaaggacaccctcatgatcagcagaacccctgaagtcacctgtgtcgtcgtggatgtcagccatgaggaccccgaggtgaaattcaactggtatgtcgatggcgtcgaggtgcacaacgccaaaaccaagcccagggaggaacagtacaactccacctacagggtggtgtccgtgctgacagtcctccaccaggactggctgaacggcaaggagtacaagtgcaaggtgtccaacaaggctctccctgcccccattgagaagaccatcagcaaggccaaaggccaacccagggagccccaggtctatacactgcctccctccagggacgaactcaccaagaaccaggtgtccctgacctgcctggtcaagggcttttatcccagcgacatcgccgtcgagtgggagtccaacggacagcccgagaataactacaagaccacccctcctgtcctcgactccgacggctccttcttcctgtacagcaagctgaccgtggacaaaagcaggtggcagcagggaaacgtgttctcctgcagcgtgatgcacgaagccctccacaaccactacacccagaaaagcctgtccctgagccccggcaaa

SEQ ID NO: 40 - protein, 448 aa, synthetic construct
EVQLVESGGGLVQPGGSLRLSCAASGFAFSSYDMSWVRQAPGKGLDWVATISGGGRYTYYPDSVKGRFTISRDNSKNNLYLQMNSLRAEDTALYYCANRYGEAWFAYWGQGTLVTVSSASTKGPSVFPLAPSSKSTSGGTAALGCLVKDYFPEPVTVSWNSGALTSGVHTFPAVLQSSGLYSLSSVVTVPSSSLGTQTYICNVNHKPSNTKVDKKVEPKSCDKTHTCPPCPAPEAAGAPSVFLFPPKPKDTLMISRTPEVTCVVVDVSHEDPEVKFNWYVDGVEVHNAKTKPREEQYNSTYRVVSVLTVLHQDWLNGKEYKCKVSNKALPAPIEKTISKAKGQPREPQVYTLPPSRDELTKNQVSLTCLVKGFYPSDIAVEWESNGQPENNYKTTPPVLDSDGSFFLYSKLTVDKSRWQQGNVFSCSVMHEALHNHYTQKSLSLSPGK

SEQ ID NO: 41 - protein, 115 aa, synthetic construct
QVQLVESGAELVKPGASMKISCKASGYSFTGYTMNWVKQAPGQCLEWIGLINPYNNITNYNQKFMGKATFTVDKSISTAYMELSRLTSDDSGVYFCARLDYRSYWGQGTLVTVSA

SEQ ID NO: 42 - protein, 110 aa, synthetic construct
QAVVTQEPSLTVSPGGTVTLTCGSSTGAVTTSNFANWVQEKPGQAFRSLIGGTNNRASWVPARFSGSLLGGKAALTISGAQPEDEAEYFCALWYSNHWVFGCGTKLTVLR

SEQ ID NO: 43 - protein, 115 aa, synthetic construct
QVQLVESGAEVKKPGASVKVSCKASGYSFTGYTMNWVRQAPGQCLEWIGLINPYNNITNYAQKFQGRVTFTVDTSISTAYMELSRLRSDDTGVYFCARLDYRSYWGQGTLVTVSA

SEQ ID NO: 44 - protein, 110 aa, synthetic construct
QAVVTQEPSLTVSPGGTVTLTCGSSTGAVTTSNFPNWVQQKPGQAPRSLIGGTNNKASWTPARFSGSLLGGKAALTISGAQPEDEAEYYCALWYSNHWVFGCGTKLTVLR

SEQ ID NO: 45 - protein, 456 aa, synthetic construct
QVQLVQSGAEVKKPGASVKVSCQASGYRFSNFVIHWVRQAPGQRFEWMGWINPYNGNKEFSAKFQDRVTFTADTSANTAYMELRSLRSADTAVYYCARVGPYSWDDSPQDNYYMDVWGKGTTVIVSSASTKGPSVFPLAPSSKSTSGGTAALGCLVKDYFPEPVTVSWNSGALTSGVHTFPAVLQSSGLYSLSSVVTVPSSSLGTQTYICNVNHKPSNTKVDKKVEPKSCDKTHTCPPCPAPELLGGPSVFLFPPKPKDTLMISRTPEVTCVVVDVSHEDPEVKFNWYVDGVEVHNAKTKPREEQYNSTYRVVSVLTVLHQDWLNGKEYKCKVSNKALPAPIEKTISKAKGQPREPQVYTLPPSREEMTKNQVSLTCLVKGFYPSDIAVEWESNGQPENNYKTTPPVLDSDGSFFLYSKLTVDKSRWQQGNVFSCSVMHEALHNHYTQKSLSLSPG

SEQ ID NO: 46 - protein, 215 aa, synthetic construct
EIVLTQSPGTLSLSPGERATFSCRSSHSIRSRRVAWYQHKPGQAPRLVIHGVSNRASGISDRFSGSGSGTDFTLTITRVEPEDFALYYCQVYGASSYTFGQGTKLERKRTVAAPSVFIFPPSDEQLKSGTASVVCLLNNFYPREAKVQWKVDNALQSGNSQESVTEQDSKDSTYSLSSTLTLSKADYEKHKVYACEVTHQGLSSPVTKSFNRGEC

SEQ ID NO: 47 - protein, 5 aa, synthetic construct
GGGGS